European Patent Specification EP 3 013 340 B9, published October 4, 2023. Title: SUBSTITUTED NUCLEOSIDES, NUCLEOTIDES AND ANALOGS THEREOF. Applicant: ALIOS BIOPHARMA, INC. Beigelman, Leonid Deval, Jerome Jin, Zhinan. The sequence listing filed with the application follows.

SEQUENCE LISTING (9 sequences)

SEQ ID NO: 1 - DNA, 17 bp, Artificial Sequence
  Synthetic Oligonucleotide
acgccactccgcacaaa

SEQ ID NO: 2 - DNA, 18 bp, Artificial Sequence
  Synthetic Oligonucleotide
gcggccagagaccacaaa

SEQ ID NO: 3 - DNA, 15 bp, Artificial Sequence
  Synthetic Oligonucleotide
agcccgggtgatgag

SEQ ID NO: 4 - DNA, 20 bp, Artificial Sequence
  Synthetic Oligonucleotide
  misc_feature 12: n = a, c, t or g
cgytggatgcgnttycatga

SEQ ID NO: 5 - DNA, 22 bp, Artificial Sequence
  Synthetic Oligonucleotide
cttagacgccatcatcattyac

SEQ ID NO: 6 - DNA, 20 bp, Artificial Sequence
  Synthetic Oligonucleotide
ggcatccacgaaactacctt

SEQ ID NO: 7 - DNA, 20 bp, Artificial Sequence
  Synthetic Oligonucleotide
agcactgtgttggcgtacag

SEQ ID NO: 8 - DNA, 20 bp, Artificial Sequence
  Synthetic Oligonucleotide
agatygcgatcycctgtcca

SEQ ID NO: 9 - DNA, 26 bp, Artificial Sequence
  Synthetic Oligonucleotide
atcatgaagtgtgacgtggacatccg